European Patent Application EP 4 372 082 A1, published May 22, 2024. Title: VARIANT POLYPEPTIDE HAVING XYLANASE ACTIVITY. Applicant: 씨제이제일제당 주식회사. The sequence listing filed with the application follows.

SEQUENCE LISTING (26 sequences)

SEQ ID NO: 1 - protein, 190 aa, synthetic construct
  REGION 1..190: note = Accession number: CAA49293
QTIQPGTGYNNGYFYSYWNDGHGGVTYTNGPGGQFSVNWSNSGNFVGGKGWQPGTKNKVINFSGSYNPNGNSYLSVYGWSRNPLIEYYIVENFGTYNPSTGATKLGEVTSDGSVYDIYRTQRVNQPSIIGTATFYQYWSVRRNHRSSGSVNTANHFNAWAQQGLTLGTMDYQIVAVEGYFSSGSASITVS

SEQ ID NO: 2 - DNA, 570 bp, synthetic construct
  source 1..570: mol_type = other DNA
cagactattcaaccaggcacaggatacaacaatggctacttctacagttactggaatgatggacacggcggtgtcacgtacaccaatggccctggcggccaattcagcgttaattggagcaacagtggtaacttcgtgggaggcaaggggtggcaaccaggcacgaaaaataaggtgataaacttttcaggttcatataatccgaatggaaacagttatctgtccgtttacggatggtcacgcaatccgctgattgaatactatatagtggagaatttcgggacctataatccctcaactggcgcgaccaaattaggcgaggtgacttcggatgggagtgtatatgacatttatagaacccaacgtgtgaaccaaccttccattataggaacggctaccttctatcaatattggtcggtacggcgtaatcacagatcgtcaggttcagtcaacacggcaaatcattttaatgcctgggctcaacaaggcttgacgcttggaacgatggactatcagatcgtagcggtggagggctatttttcgagtgggtctgcgagcataacggtcagc

SEQ ID NO: 3 - DNA, 32 bp, synthetic construct
  source 1..32: mol_type = other DNA
caaccaggcacaggatacaacaatggctactt

SEQ ID NO: 4 - DNA, 45 bp, synthetic construct
  source 1..45: mol_type = other DNA
tgtgcctggttgmnnagtctgcatatggatatctcctttttccag

SEQ ID NO: 5 - protein, 190 aa, synthetic construct
QCTQPGTGYNNGYFYSYWNDGHGGVTYCNGPGGQFSVDWSNSGNFVGGKGWQPGTRNKVINYSGTYNPNGNSYLSVYGWTRNPLIEYYIVENYGTYNPSTGATKLGEVTSDGSTYDIYRTQRVNQPSIIGTATFYQYWSVRRNKRTSGTVTTANHFNAWARQGLVLGTMDYQIVAVEGYFSSGSASITVS

SEQ ID NO: 6 - DNA, 570 bp, synthetic construct
  source 1..570: mol_type = other DNA
cagtgtactcaacctggtacagggtacaataatggttacttttacagctactggaatgatgggcacggtggtgttacctactgtaatggaccaggaggccagtttagtgtagactggagcaacagtggaaatttcgttgggggcaaggggtggcagcccggaactcgcaataaggtgattaactacagtgggacttacaacccaaatggcaattcgtatctgtcagtgtatggatggacccgtaatcccttaatagaatactacattgtcgaaaattatggaacatataacccatcgactggagcaaccaaacttggggaagtcacctcagatggatcgacatacgatatatatcgtacacagagagtcaaccagccctcaataataggcacagccacgttctatcagtattggagtgtacgtcgtaacaagcgcacatctggtactgtaacaactgcgaaccacttcaacgcctgggctcggcaggggttggtgttggggaccatggactatcagatagttgcagtagaagggtatttctcctctggttccgcttcgataacagtttcg

SEQ ID NO: 7 - DNA, 30 bp, synthetic construct
  source 1..30: mol_type = other DNA
caacctggtacagggtacaataatggttac

SEQ ID NO: 8 - DNA, 45 bp, synthetic construct
  source 1..45: mol_type = other DNA
tgtaccaggttgaatacactgcatatgtatatctccttcttaaag

SEQ ID NO: 9 - DNA, 30 bp, synthetic construct; identical to SEQ ID NO: 7
  source 1..30: mol_type = other DNA

SEQ ID NO: 10 - DNA, 45 bp, synthetic construct
  source 1..45: mol_type = other DNA
tgtaccaggttgcacacactgcatatgtatatctccttcttaaag

SEQ ID NO: 11 - DNA, 31 bp, synthetic construct
  source 1..31: mol_type = other DNA
aataaggtgattaactacagtgggacttaca

SEQ ID NO: 12 - DNA, 32 bp, synthetic construct
  source 1..32: mol_type = other DNA
aatcaccttatttttagttccgggctgccacc

SEQ ID NO: 13 - DNA, 24 bp, synthetic construct
  source 1..24: mol_type = other DNA
agtgggacttacaacccaaatggc

SEQ ID NO: 14 - DNA, 35 bp, synthetic construct
  source 1..35: mol_type = other DNA
gtaagtcccactaaagttaatcaccttattgcgag

SEQ ID NO: 15 - DNA, 26 bp, synthetic construct
  source 1..26: mol_type = other DNA
tctggtactgtaacaactgcgaacca

SEQ ID NO: 16 - DNA, 32 bp, synthetic construct
  source 1..32: mol_type = other DNA
tacagtaccagaagagcgcttgttacgacgta

SEQ ID NO: 17 - protein, 190 aa, synthetic construct
QCIQPGTGYNNGYFYSYWNDGHGGVTYCNGPGGQFSVDWSNSGNFVGGKGWQPGTRNKVINYSGTYNPNGNSYLSVYGWTRNPLIEYYIVENYGTYNPSTGATKLGEVTSDGSTYDIYRTQRVNQPSIIGTATFYQYWSVRRNKRTSGTVTTANHFNAWARQGLVLGTMDYQIVAVEGYFSSGSASITVS

SEQ ID NO: 18 - DNA, 570 bp, synthetic construct
  source 1..570: mol_type = other DNA
cagtgtattcaacctggtacagggtacaataatggttacttttacagctactggaatgatgggcacggtggtgttacctactgtaatggaccaggaggccagtttagtgtagactggagcaacagtggaaatttcgttgggggcaaggggtggcagcccggaactcgcaataaggtgattaactacagtgggacttacaacccaaatggcaattcgtatctgtcagtgtatggatggacccgtaatcccttaatagaatactacattgtcgaaaattatggaacatataacccatcgactggagcaaccaaacttggggaagtcacctcagatggatcgacatacgatatatatcgtacacagagagtcaaccagccctcaataataggcacagccacgttctatcagtattggagtgtacgtcgtaacaagcgcacatctggtactgtaacaactgcgaaccacttcaacgcctgggctcggcaggggttggtgttggggaccatggactatcagatagttgcagtagaagggtatttctcctctggttccgcttcgataacagtttcg

SEQ ID NO: 19 - protein, 190 aa, synthetic construct
QCVQPGTGYNNGYFYSYWNDGHGGVTYCNGPGGQFSVDWSNSGNFVGGKGWQPGTRNKVINYSGTYNPNGNSYLSVYGWTRNPLIEYYIVENYGTYNPSTGATKLGEVTSDGSTYDIYRTQRVNQPSIIGTATFYQYWSVRRNKRTSGTVTTANHFNAWARQGLVLGTMDYQIVAVEGYFSSGSASITVS

SEQ ID NO: 20 - DNA, 570 bp, synthetic construct
  source 1..570: mol_type = other DNA
cagtgtgtgcaacctggtacagggtacaataatggttacttttacagctactggaatgatgggcacggtggtgttacctactgtaatggaccaggaggccagtttagtgtagactggagcaacagtggaaatttcgttgggggcaaggggtggcagcccggaactcgcaataaggtgattaactacagtgggacttacaacccaaatggcaattcgtatctgtcagtgtatggatggacccgtaatcccttaatagaatactacattgtcgaaaattatggaacatataacccatcgactggagcaaccaaacttggggaagtcacctcagatggatcgacatacgatatatatcgtacacagagagtcaaccagccctcaataataggcacagccacgttctatcagtattggagtgtacgtcgtaacaagcgcacatctggtactgtaacaactgcgaaccacttcaacgcctgggctcggcaggggttggtgttggggaccatggactatcagatagttgcagtagaagggtatttctcctctggttccgcttcgataacagtttcg

SEQ ID NO: 21 - protein, 190 aa, synthetic construct
QCTQPGTGYNNGYFYSYWNDGHGGVTYCNGPGGQFSVDWSNSGNFVGGKGWQPGTKNKVINYSGTYNPNGNSYLSVYGWTRNPLIEYYIVENYGTYNPSTGATKLGEVTSDGSTYDIYRTQRVNQPSIIGTATFYQYWSVRRNKRTSGTVTTANHFNAWARQGLVLGTMDYQIVAVEGYFSSGSASITVS

SEQ ID NO: 22 - DNA, 570 bp, synthetic construct
  source 1..570: mol_type = other DNA
cagtgtactcaacctggtacagggtacaataatggttacttttacagctactggaatgatgggcacggtggtgttacctactgtaatggaccaggaggccagtttagtgtagactggagcaacagtggaaatttcgttgggggcaaggggtggcagcccggaactaaaaataaggtgattaactacagtgggacttacaacccaaatggcaattcgtatctgtcagtgtatggatggacccgtaatcccttaatagaatactacattgtcgaaaattatggaacatataacccatcgactggagcaaccaaacttggggaagtcacctcagatggatcgacatacgatatatatcgtacacagagagtcaaccagccctcaataataggcacagccacgttctatcagtattggagtgtacgtcgtaacaagcgcacatctggtactgtaacaactgcgaaccacttcaacgcctgggctcggcaggggttggtgttggggaccatggactatcagatagttgcagtagaagggtatttctcctctggttccgcttcgataacagtttcg

SEQ ID NO: 23 - protein, 190 aa, synthetic construct
QCTQPGTGYNNGYFYSYWNDGHGGVTYCNGPGGQFSVDWSNSGNFVGGKGWQPGTRNKVINFSGTYNPNGNSYLSVYGWTRNPLIEYYIVENYGTYNPSTGATKLGEVTSDGSTYDIYRTQRVNQPSIIGTATFYQYWSVRRNKRTSGTVTTANHFNAWARQGLVLGTMDYQIVAVEGYFSSGSASITVS

SEQ ID NO: 24 - DNA, 570 bp, synthetic construct
  source 1..570: mol_type = other DNA
cagtgtactcaacctggtacagggtacaataatggttacttttacagctactggaatgatgggcacggtggtgttacctactgtaatggaccaggaggccagtttagtgtagactggagcaacagtggaaatttcgttgggggcaaggggtggcagcccggaactcgcaataaggtgattaactttagtgggacttacaacccaaatggcaattcgtatctgtcagtgtatggatggacccgtaatcccttaatagaatactacattgtcgaaaattatggaacatataacccatcgactggagcaaccaaacttggggaagtcacctcagatggatcgacatacgatatatatcgtacacagagagtcaaccagccctcaataataggcacagccacgttctatcagtattggagtgtacgtcgtaacaagcgcacatctggtactgtaacaactgcgaaccacttcaacgcctgggctcggcaggggttggtgttggggaccatggactatcagatagttgcagtagaagggtatttctcctctggttccgcttcgataacagtttcg

SEQ ID NO: 25 - protein, 190 aa, synthetic construct
QCTQPGTGYNNGYFYSYWNDGHGGVTYCNGPGGQFSVDWSNSGNFVGGKGWQPGTRNKVINYSGTYNPNGNSYLSVYGWTRNPLIEYYIVENYGTYNPSTGATKLGEVTSDGSTYDIYRTQRVNQPSIIGTATFYQYWSVRRNKRSSGTVTTANHFNAWARQGLVLGTMDYQIVAVEGYFSSGSASITVS

SEQ ID NO: 26 - DNA, 570 bp, synthetic construct
  source 1..570: mol_type = other DNA
cagtgtactcaacctggtacagggtacaataatggttacttttacagctactggaatgatgggcacggtggtgttacctactgtaatggaccaggaggccagtttagtgtagactggagcaacagtggaaatttcgttgggggcaaggggtggcagcccggaactcgcaataaggtgattaactacagtgggacttacaacccaaatggcaattcgtatctgtcagtgtatggatggacccgtaatcccttaatagaatactacattgtcgaaaattatggaacatataacccatcgactggagcaaccaaacttggggaagtcacctcagatggatcgacatacgatatatatcgtacacagagagtcaaccagccctcaataataggcacagccacgttctatcagtattggagtgtacgtcgtaacaagcgctcttctggtactgtaacaactgcgaaccacttcaacgcctgggctcggcaggggttggtgttggggaccatggactatcagatagttgcagtagaagggtatttctcctctggttccgcttcgataacagtttcg